European Patent Specification EP 3 792 363 B1, published June 26, 2024. Title: method and kit for identifying lung cancer status. Applicant: EXELLON MEDICAL TECHNOLOGY. The sequence listing filed with the application follows.

SEQUENCE LISTING (101 sequences)

SEQ ID NO: 1 - DNA, 279 bp, Homo sapiens
cggacaaaaccataagtagttaccttcattgttccgtcggccacgagggaagctcgagctgagcggagggcagatcccaagggtcgtagcccctggccgtgtggaccgggtctgcggctgcagagcgcggtcccggctgcagcaagacctggggcagtgcccgaggcggcggcgagtacacgtggcgggctggattgcagaccggccctctcgcggcggagactcgcgacctagcggattgcatcagcaggaagacactaaggctgctcccccaggccg

SEQ ID NO: 2 - DNA, 360 bp, Homo sapiens
attcgaacccagtggaatcagaaccgtgcaggtcccataacccacctagaccctagcaactccaggctagagggtcaccgcgtctatgcgaggccgggtgggcgggccgtcagctccgccctggggaggggtccgcgctgctgattggctgtggccggcaggtgaaccctcagccaatcagcggtacggggggcggtgcctccggggctcacctggctgcagccacgcaccccctctcagtggcgtcggaactgcaaagcacctgtgagcttgcggaagtcagttcagactccagcccgctccagcccggcccgacccgaccgcacccggcgcctgccctcgctcggcgtccccggccag

SEQ ID NO: 3 - DNA, 690 bp, Homo sapiens
gaggtttaggggtgtagtcaagccagatgcaccgaggttgctgcggtgggaagagggcgctgggagggaggaggacctggggcgcagccgtggtgggtgcgccctgccaagaagggcgggggcgacggggcgcgcacgcggaggaggaggaggaggagggagacgggagggcgtgtgagcgagtgagacaagaaaagggagcgcgcccgccgccgccgccgccgccgccctcctctggagagagaggctggagtgaggctgtgcgaagcgccgcatttcaatgaggacgggccgaggcacatccctgcactagtggccgcaaccgaggcgccgcgctccagcagctgctgccgcccagcccggccccgccgccgccccccagccctgcagccccgcagccccggccgcgcccagcccggcgaggacagcaccaggaggcggcccccagcgcggccacaaagacccccggcggcgtctctccgcggaccggtgcgtggtttgccttccctggggacgggagctgcggggagggcggccgggggactccgcagagcccgctccgcccgcagccgcggggcgccgagggcagggcgggcgctcagcttggccccgccgccccgcccgcagttcctcgaaaggcggccgccctgccctggccagcctggcccgacccgggggcgttgcgtgcgg

SEQ ID NO: 4 - DNA, 475 bp, Homo sapiens
tgcggggaaaggttttttaaaactcggtttcatactattattattactaaggacaaccgggcaggctgaggtcccaacgtggatgatccgagttggcctcgcgccggggctctgcagccactgccctgtgcgctcagcacctctgggggcgatcagggcccctgcgcttccgcccgccgcccggcagtcgagagcaccctgtgcccagactggccgactcattctcccccgaattttgtttagagctggcaagggggacttagctcgcgccccaagacctgggcttgcagcgccgccaacaggcccggggacacgaggcgctccaggccggggtcttcccggctgctggcccctctcgctccccacccgctggcggcgcctcggtcgcccgcaattgacccaacccgcttcctgcgtttgcccctcaggtttcccgtttctccacaaaggcctaggggagcctcgcccacaggct

SEQ ID NO: 5 - DNA, 353 bp, Homo sapiens
aggtttaatgccataaggccggctggagggcaagcccgcgaaggagagcgcaccgggcgtgggctccagccaggagcgcatgtacctgccgtccggcgccgccgccgccacgggcgcctgggggtgcacgtaggggtggtggtgatggtggtggtacaccgcagcgggtacagcgttggcgcccgccgcgtgcactgggttccacgaggcgccaaacaccgtcgccttggactggaagctgcacgggctgaagtcggggtgctcggccagcgtcgccgcctgccggggaggctggcccagggtccccggcgcatagcggccaacgctcagctcatccgcggcgtcggcgccca

SEQ ID NO: 6 - DNA, 450 bp, Homo sapiens
cttcttcagcctgtccggcctcagcatcatctgcgccatgagtgtcgagcgctacctggccatcaaccatgcctatttctacagccactacgtggacaagcgattggcgggcctcacgctctttgcagtctatgcgtccaacgtgctcttttgcgcgctgcccaacatgggtctcggtagctcgcggctgcagtacccagacacctggtgcttcatcgactggaccaccaacgtgacggcgcacgccgcctactcctacatgtacgcgggcttcagctccttcctcattctcgccaccgtcctctgcaacgtgcttgtgtgcggcgcgctgctccgcatgcaccgccagttcatgcgccgcacctcgctgggcaccgagcagcaccacgcggccgcggccgcctcggttgcctcccggggccaccccgctgcctccccagccttgccgcg

SEQ ID NO: 7 - DNA, 828 bp, Homo sapiens
acagacagaaaggcgcacagaggaatttaaagtgtgggctggggggcgaggcggtgggcgggaggcgagcgggcgcaggcggaacaccgttttccaagctaagccgccgcaaataaaaaggcgtaaagggagagaagttggtgctcaacgtgagccaggagcagcgtcccggctcctcccctgctcattttaaaagcacttcttgtattgtttttaaggtgagaaataggaaagaaaacgccggcttgtgcgctcgctgcctgcctctctggctgtctgcttttgcagggctgctgggagtttttaagctctgtgagaatcctgggagttggtgatgtcagactagttgggtcatttgaaggttagcagcccgggtagggttcaccgaaagttcactcgcatatattaggcaattcaatctttcattctgtgtgacagaagtagtaggaagtgagctgttcagaggcaggagggtctattctttgccaaaggggggaccagaattcccccatgcgagctgtttgaggactgggatgccgagaacgcgagcgatccgagcagggtttgtctgggcaccgtcggggtaggatccggaacgcattcggaaggctttttgcaagcatttacttggaaggagaacttgggatctttctgggaaccccccgccccggctggattggccgagcaagcctggaaaatggtaaatgatcatttggatcaattacaggcttttagctggcttgtctgtcataattcatgattcggggctgggaaaaagaccaacagcctacgtgccaaaaaaggggcagagtttgatggagttgggtg

SEQ ID NO: 8 - DNA, 443 bp, Homo sapiens
ctgcgagagcgcgcccagccccgccttcgggccccacagtccctgcacccaggtttccattgcgcggctctcctcagctccttcccgccgcccagtctggatcctgggggaggcgctgaagtcggggcccgccctgtggccccgcccggcccgcgcttgctagcgcccaaagccagcgaagcacgggcccaaccgggccatgtcgggggagcctgagctcattgagctgcgggagctggcacccgctgggcgcgctgggaagggccgcacccggctggagcgtgccaacgcgctgcgcatcgcgcggggcaccgcgtgcaaccccacacggcagctggtccctggccgtggccaccgcttccagcccgcggggcccgccacgcacacgtggtgcgacctctgtggcgacttcatctggggcgtcgtgcgcaaaggcctgcagt

SEQ ID NO: 9 - DNA, 572 bp, Homo sapiens
cggtgcgggtgcgggaacctgatccgcccgggaggcgggggcggggcgggggcgcagcgcgcggggaggggccggcgcccgccttcctcccccattcattcagctgagccagggggcctaggggctcctccggcggctagctctgcactgcaggagcgcgggcgcggcgccccagccagcgcgcagggcccgggccccgccgggggcgcttcctcgccgctgccctccgcgcgacccgctgcccaccagccatcatgtcggaccccgcggtcaacgcgcagctggatgggatcatttcggacttcgaaggtgggtgctgggctggctgctgcggccgcggacgtgctggagaggaccctgcgggtgggcctggcgcgggacgggggtgcgctgaggggagacgggagtgcgctgaggggagacgggacccctaatccaggcgccctcccgctgagagcgccgcgcgcccccggccccgtgcccgcgccgcctacgtgggggaccctgttaggggcacccgcgtagaccctgcgcgccctcacaggaccctgtgctcgttctgcgcactgccg

SEQ ID NO: 10 - DNA, 490 bp, Homo sapiens
tggctctctgcctaccgcaaacttgctggtctaatttaggaacaattgggccgaaaggtatcagcgagagcaacagaccccggtgttgtgccgcacagggagccgcatccgcagacgcccctcgctgcccctgggctcgggccaaaccctgcataaggtcccctggacagccaggtaatctccgtcccgcctgcccgaccggggtcgcacgagcacaggcgcccacgccatgttggctgcccaaagggctcgccgcccaagccgggccagaaggcaggaggcggaaaaccagcctccggtggcgggcgaaagcaaccgctctttctgttctctcttcgccctccctcgtggaaacgcagactcgaccctaaacgcttaacccacagagatcaacaggttcaagcggaatattcgcgatcctcggtttctattggttgctcaaagccttttcatgcaaccagcagctcggatgtttaataaaatatgaatt

SEQ ID NO: 11 - DNA, 24 bp, artificial sequence
tgttgatgtaattcgttaggtcgc

SEQ ID NO: 12 - DNA, 19 bp, artificial sequence
aatacccgaaacgacgacg

SEQ ID NO: 13 - DNA, 32 bp, artificial sequence
atttgttaggttgtgagtttttgttgtgagag

SEQ ID NO: 14 - DNA, 22 bp, artificial sequence
aaaccgaccctctcgcgacgaa

SEQ ID NO: 15 - DNA, 21 bp, artificial sequence
tttattgtttcgtcggttacg

SEQ ID NO: 16 - DNA, 20 bp, artificial sequence
cccaaatcttactacaaccg

SEQ ID NO: 17 - DNA, 31 bp, artificial sequence
tgttggttatgagggaagtttgagttgagtg

SEQ ID NO: 18 - DNA, 23 bp, artificial sequence
cgcgctctacaaccgcaaacccg

SEQ ID NO: 19 - DNA, 25 bp, artificial sequence
cgaatttagtggaattagaatcgtg

SEQ ID NO: 20 - DNA, 19 bp, artificial sequence
cgaaactaacgacccgccc

SEQ ID NO: 21 - DNA, 29 bp, artificial sequence
caaaactaacaacccacccacccaacctc

SEQ ID NO: 22 - DNA, 27 bp, artificial sequence
cccgacctcgcataaacgcgataaccc

SEQ ID NO: 23 - DNA, 18 bp, artificial sequence
ttggggaggggttcgcgt

SEQ ID NO: 24 - DNA, 25 bp, artificial sequence
cgacgccactaaaaaaaaatacgta

SEQ ID NO: 25 - DNA, 27 bp, artificial sequence
gaggggtttgtgttgttgattggttgt

SEQ ID NO: 26 - DNA, 31 bp, artificial sequence
ttaactaaaaattcacctaccgaccacaacc

SEQ ID NO: 27 - DNA, 17 bp, artificial sequence
tgcggtgggaagagggc

SEQ ID NO: 28 - DNA, 17 bp, artificial sequence
cacgccctcccgtctcc

SEQ ID NO: 29 - DNA, 23 bp, artificial sequence
tggtgggaagagggtgttgggag

SEQ ID NO: 30 - DNA, 24 bp, artificial sequence
acccaccacgactacgccccaaat

SEQ ID NO: 31 - DNA, 22 bp, artificial sequence
tagtttcggtcgcgtttagttc

SEQ ID NO: 32 - DNA, 19 bp, artificial sequence
tctacgaaatcccccgacc

SEQ ID NO: 33 - DNA, 34 bp, artificial sequence
ttggttgtgtttagtttggtgaggatagtattag

SEQ ID NO: 34 - DNA, 22 bp, artificial sequence
accgcgctaaaaaccgcctcct

SEQ ID NO: 35 - DNA, 18 bp, artificial sequence
gggtaaacgtaggaagcg

SEQ ID NO: 36 - DNA, 18 bp, artificial sequence
gactactaacccctctcg

SEQ ID NO: 37 - DNA, 30 bp, artificial sequence
tgtaggaagtgggttgggttaattgtgggt

SEQ ID NO: 38 - DNA, 21 bp, artificial sequence
ccgctaacgacgcctcgatcg

SEQ ID NO: 39 - DNA, 18 bp, artificial sequence
cgggaagatttcggtttg

SEQ ID NO: 40 - DNA, 19 bp, artificial sequence
ccccaaaacctaaacttac

SEQ ID NO: 41 - DNA, 33 bp, artificial sequence
ttttggtttggagcgttttgtgtttttgggttt

SEQ ID NO: 42 - DNA, 20 bp, artificial sequence
cgccgccaacaaacccgaaa

SEQ ID NO: 43 - DNA, 19 bp, artificial sequence
tagggtgttttcgattgtc

SEQ ID NO: 44 - DNA, 19 bp, artificial sequence
ccaacgtaaataatccgaa

SEQ ID NO: 45 - DNA, 27 bp, artificial sequence
tttgattgttgggtggtgggtggaagt

SEQ ID NO: 46 - DNA, 24 bp, artificial sequence
cgcgccgaaactctacaaccacta

SEQ ID NO: 47 - DNA, 23 bp, artificial sequence
gggttttagttaggagcgtatgt

SEQ ID NO: 48 - DNA, 20 bp, artificial sequence
ccatcaccaccacccctacg

SEQ ID NO: 49 - DNA, 34 bp, artificial sequence
gagtgtatgtatttgttgtttggtgttgttgttg

SEQ ID NO: 50 - DNA, 23 bp, artificial sequence
cgcccgtaacgacgacgacgccg

SEQ ID NO: 51 - DNA, 18 bp, artificial sequence
gatggtggtggtatatcg

SEQ ID NO: 52 - DNA, 18 bp, artificial sequence
acgatatttaacgcctcg

SEQ ID NO: 53 - DNA, 25 bp, artificial sequence
gtggtatattgtagtgggtatagtg

SEQ ID NO: 54 - DNA, 21 bp, artificial sequence
cgcgacgaacgccaacgctat

SEQ ID NO: 55 - DNA, 25 bp, artificial sequence
ttagatatttggtgttttatcgatt

SEQ ID NO: 56 - DNA, 22 bp, artificial sequence
aaaaactaaaacccgcgtacat

SEQ ID NO: 57 - DNA, 38 bp, artificial sequence
ttttattgattggattattaatgtgatggtgtatgttg

SEQ ID NO: 58 - DNA, 28 bp, artificial sequence
ataaacgacgtacgccgtcacgttaata

SEQ ID NO: 59 - DNA, 24 bp, artificial sequence
tgggtattgtagtcgcgagttatc

SEQ ID NO: 60 - DNA, 22 bp, artificial sequence
ctacgtaaacaaacgattaacg

SEQ ID NO: 61 - DNA, 32 bp, artificial sequence
tgtgagttattgagatttatgttgggtagtgt

SEQ ID NO: 62 - DNA, 35 bp, artificial sequence
caatctatacgtccaacgtactcttttacgcgcta

SEQ ID NO: 63 - DNA, 25 bp, artificial sequence
gcgtatagaggaatttaaagtgtgg

SEQ ID NO: 64 - DNA, 27 bp, artificial sequence
acgcctttttatttacgacgacttaac

SEQ ID NO: 65 - DNA, 39 bp, artificial sequence
ttatttacaacaacttaacttaaaaaacaatattccacc

SEQ ID NO: 66 - DNA, 21 bp, artificial sequence
tattccgcctacgcccgctcg

SEQ ID NO: 67 - DNA, 27 bp, artificial sequence
gaatttttttatgcgagttgtttgagg

SEQ ID NO: 68 - DNA, 25 bp, artificial sequence
ttccgaatacgttccgaatcctacc

SEQ ID NO: 69 - DNA, 33 bp, artificial sequence
ttatgtgagttgtttgaggattgggatgttgag

SEQ ID NO: 70 - DNA, 26 bp, artificial sequence
aacaaaccctactcgaatcgctcgcg

SEQ ID NO: 71 - DNA, 21 bp, artificial sequence
tgggaatttttcgtttcggtt

SEQ ID NO: 72 - DNA, 29 bp, artificial sequence
acacgtaaactattaatctttttcccaac

SEQ ID NO: 73 - DNA, 34 bp, artificial sequence
cataaactattaatctttttcccaaccccaaatc

SEQ ID NO: 74 - DNA, 30 bp, artificial sequence
tcatttaccattttccaaacttactcgacc

SEQ ID NO: 75 - DNA, 19 bp, artificial sequence
gcgttgaagtcggggttcg

SEQ ID NO: 76 - DNA, 19 bp, artificial sequence
ccgattaaacccgtacttc

SEQ ID NO: 77 - DNA, 33 bp, artificial sequence
ttggggtttgttttgtggtttcgtttggtttgt

SEQ ID NO: 78 - DNA, 20 bp, artificial sequence
cgctaacaaacgcgaaccga

SEQ ID NO: 79 - DNA, 19 bp, artificial sequence
gggagtttgagtttattga

SEQ ID NO: 80 - DNA, 21 bp, artificial sequence
gatacgcaacgcgttaacacg

SEQ ID NO: 81 - DNA, 33 bp, artificial sequence
cacattaacacactccaaccaaatacaaccctt

SEQ ID NO: 82 - DNA, 21 bp, artificial sequence
cgcccaacgaataccaactcc

SEQ ID NO: 83 - DNA, 20 bp, artificial sequence
cgcgattcgttgtttattag

SEQ ID NO: 84 - DNA, 18 bp, artificial sequence
caccttcgaaatccgaaa

SEQ ID NO: 85 - DNA, 36 bp, artificial sequence
aaaatccaaaataatcccatccaactacacattaac

SEQ ID NO: 86 - DNA, 27 bp, artificial sequence
cgcgttaaccgcgaaatccgacataat

SEQ ID NO: 87 - DNA, 19 bp, artificial sequence
tagcgtattttcgtttcgc

SEQ ID NO: 88 - DNA, 25 bp, artificial sequence
cgaacttcgaaaataaatactaaac

SEQ ID NO: 89 - DNA, 32 bp, artificial sequence
tttgttttgtgttaggtttatttgtagggttt

SEQ ID NO: 90 - DNA, 22 bp, artificial sequence
aactactacgaccgcgaacgta

SEQ ID NO: 91 - DNA, 18 bp, artificial sequence
gttcgtgcgatttcggtc

SEQ ID NO: 92 - DNA, 19 bp, artificial sequence
tcgctacccctaaactcga

SEQ ID NO: 93 - DNA, 25 bp, artificial sequence
tgattttggttgggtaggtgggatg

SEQ ID NO: 94 - DNA, 23 bp, artificial sequence
caaccaaataatctccgtcccgc

SEQ ID NO: 95 - DNA, 17 bp, artificial sequence
ggcgggcgaaagtaatc

SEQ ID NO: 96 - DNA, 20 bp, artificial sequence
cgaaaatcgcgaatattccg

SEQ ID NO: 97 - DNA, 43 bp, artificial sequence
acaaatattccacttaaacctattaatctctataaattaaaca

SEQ ID NO: 98 - DNA, 27 bp, artificial sequence
aaaatcgaatctacgtttccacgaaaa

SEQ ID NO: 99 - DNA, 23 bp, artificial sequence
gtgatggaggaggtttagtaagt

SEQ ID NO: 100 - DNA, 23 bp, artificial sequence
ccaataaaacctactcctccctt

SEQ ID NO: 101 - DNA, 30 bp, artificial sequence
accaccacccaacacacaataacaaacaca